European Patent Specification EP 3 320 084 B9, published October 4, 2023. Title: DEVELOPMENT OF AN ASPARAGINE-REDUCING YEAST BY ADAPTIVE EVOLUTION AND USES THEREOF TO REDUCE ACRYLAMIDE FORMATION. Applicant: Renaissance BioScience Corp. The sequence listing filed with the application follows.

SEQUENCE LISTING (8 sequences)

SEQ ID NO: 1 - DNA, 19 bp, Artificial Sequence
  Synthetic Primer
tcaacaatggaatcccaac

SEQ ID NO: 2 - DNA, 20 bp, Artificial Sequence
  Synthetic Primer
catcttaacaccgtatatga

SEQ ID NO: 3 - DNA, 21 bp, Artificial Sequence
  Synthetic Primer
gagcggatgaacagggatatt

SEQ ID NO: 4 - DNA, 20 bp, Artificial Sequence
  Synthetic Primer
gggtctgtgaggttggaaat

SEQ ID NO: 5 - DNA, 22 bp, Artificial Sequence
  Synthetic Primer
caaactgagagtggacggtaag

SEQ ID NO: 6 - DNA, 21 bp, Artificial Sequence
  Synthetic Primer
gttgactatagctggcggaaa

SEQ ID NO: 7 - DNA, 22 bp, Artificial Sequence
  Synthetic Primer
cgtctggattggtggttctatc

SEQ ID NO: 8 - DNA, 22 bp, Artificial Sequence
  Synthetic Primer
ggaccactttcgtcgtattctt